European Patent Application EP 4 230 656 A1, published August 23, 2023. Title: ANTI-TROP-2 ANTIBODY, ANTIGEN-BINDING FRAGMENT THEREOF OR MUTANT THEREOF, AND MEDICAL USE THEREOF. Applicant: SHANGHAI HANSOH BIOMEDICAL CO., LTD. JIANGSU HANSOH PHARMACEUTICAL GROUP CO., LTD. Application PCT/CN2021/123731. The sequence listing filed with the application follows.

SEQUENCE LISTING (43 sequences)

SEQ ID NO: 1 - protein, 331 aa, Homo sapiens
MARGPGLAPPPLRLPLLLLVLAAVTGHTAAQDNCTCPTNKMTVCSPDGPGGRCQCRALGSGMAVDCSTLTSKCLLLKARMSAPKNARTLVRPSEHALVDNDGLYDPDCDPEGRFKARQCNQTSVCWCVNSVGVRRTDKGDLSLRCDELVRTHHILIDLRHRPTAGAFNHSDLDAELRRLFRERYRLHPKFVAAVHYEQPTIQIELRQNTSQKAAGDVDIGDAAYYFERDIKGESLFQGRGGLDLRVRGEPLQVERTLIYYLDEIPPKFSMKRLTAGLIAVIVVVVVALVAGMAVLVITNRRKSGKYKKVEIKELGELRKEPSLHHHHHHHH

SEQ ID NO: 2 - protein, 121 aa, Mus musculus
QVQLQQPGAELVRPGASVKLSCRASGYTFTNYWMNWVKQRPEQGLEWIGRIDPNDSETHYNQKFKDRAILTVDKASNTAYMQLSGLTSEDSAVHYCARSGFGSTYWFFDVWGAGTTVTVSS

SEQ ID NO: 3 - protein, 107 aa, Mus musculus
DIVMTQSHKFMSTSVGDRVSITCKASQDVSTAVAWYQQKPGQSPKLLIYSASYRYTGVPDRFAGSGYGTDFTFTISSVQTEDLTVYHCQQHYSTPLTFGPGTRLELK

SEQ ID NO: 4 - protein, 5 aa, Mus musculus
NYWMN

SEQ ID NO: 5 - protein, 17 aa, Mus musculus
RIDPNDSETHYNQKFKD

SEQ ID NO: 6 - protein, 12 aa, Mus musculus
SGFGSTYWFFDV

SEQ ID NO: 7 - protein, 11 aa, Mus musculus
KASQDVSTAVA

SEQ ID NO: 8 - protein, 7 aa, Mus musculus
SASYRYT

SEQ ID NO: 9 - protein, 9 aa, Mus musculus
QQHYSTPLT

SEQ ID NO: 10 - protein, 121 aa, Artificial Sequence
  DOMAIN: Variable region
EVQLLESGGGLVQPGGSLRLSCAASGFTVSNYWMNWVRQAPGKGLEWMGRIDPNDSETHYNQKFKDRVTISVDKSKNQFSLKLSSVTAADTAVYYCARSGFGSTYWFFDVWGQGTTVTVSS

SEQ ID NO: 11 - protein, 107 aa, Artificial Sequence
  DOMAIN: Variable region
DVVMTQSPLSLPVTLGQPASISCKASQDVSTAVAWYQQKPGKAPKLFIYSASYRYTGVPSRFSGSGSGTDFTLTISSLQPEDFATYYCQQHYSTPLTFGQGTRLEIK

SEQ ID NO: 12 - protein, 330 aa, Homo sapiens [sequence omitted]

SEQ ID NO: 13 - protein, 107 aa, Homo sapiens [sequence omitted]

SEQ ID NO: 14 - protein, 451 aa, Artificial Sequence
  CHAIN: Heavy chain
EVQLLESGGGLVQPGGSLRLSCAASGFTVSNYWMNWVRQAPGKGLEWMGRIDPNDSETHYNQKFKDRVTISVDKSKNQFSLKLSSVTAADTAVYYCARSGFGSTYWFFDVWGQGTTVTVSSASTKGPSVFPLAPSSKSTSGGTAALGCLVKDYFPEPVTVSWNSGALTSGVHTFPAVLQSSGLYSLSSVVTVPSSSLGTQTYICNVNHKPSNTKVDKKVEPKSCDKTHTCPPCPAPELLGGPSVFLFPPKPKDTLMISRTPEVTCVVVDVSHEDPEVKFNWYVDGVEVHNAKTKPREEQYNSTYRVVSVLTVLHQDWLNGKEYKCKVSNKALPAPIEKTISKAKGQPREPQVYTLPPSRDELTKNQVSLTCLVKGFYPSDIAVEWESNGQPENNYKTTPPVLDSDGSFFLYSKLTVDKSRWQQGNVFSCSVMHEALHNHYTQKSLSLSPGK

SEQ ID NO: 15 - protein, 214 aa, Artificial Sequence
  CHAIN: Light chain
DVVMTQSPLSLPVTLGQPASISCKASQDVSTAVAWYQQKPGKAPKLFIYSASYRYTGVPSRFSGSGSGTDFTLTISSLQPEDFATYYCQQHYSTPLTFGQGTRLEIKRTVAAPSVFIFPPSDEQLKSGTASVVCLLNNFYPREAKVQWKVDNALQSGNSQESVTEQDSKDSTYSLSSTLTLSKADYEKHKVYACEVTHQGLSSPVTKSFNRGEC

SEQ ID NO: 16 - protein, 121 aa, Artificial Sequence
  DOMAIN: Variable region
EVQLLESGGGLVQPGGSLRLSCAASGFTVSNYWMNWVRQAPGKGLEWMGRIDPRDSETHYNQKFKDRVTISVDKSKNQFSLKLSSVTAADTAVYYCARSGFGSTYWFFDVWGQGTTVTVSS

SEQ ID NO: 17 - protein, 121 aa, Artificial Sequence
  DOMAIN: Variable region
EVQLLESGGGLVQPGGSLRLSCAASGFTVSNYWMNWVRQAPGKGLEWMGRIDPYDSETHYNQKFKDRVTISVDKSKNQFSLKLSSVTAADTAVYYCARSGFGSTYWFFDVWGQGTTVTVSS

SEQ ID NO: 18 - protein, 121 aa, Artificial Sequence
  DOMAIN: Variable region
EVQLLESGGGLVQPGGSLRLSCAASGFTVSNYWMNWVRQAPGKGLEWMGRIDPQDSETHYNQKFKDRVTISVDKSKNQFSLKLSSVTAADTAVYYCARSGFGSTYWFFDVWGQGTTVTVSS

SEQ ID NO: 19 - protein, 121 aa, Artificial Sequence
  DOMAIN: Variable region
EVQLLESGGGLVQPGGSLRLSCAASGFTVSNYWMNWVRQAPGKGLEWMGRIDPLDSETHYNQKFKDRVTISVDKSKNQFSLKLSSVTAADTAVYYCARSGFGSTYWFFDVWGQGTTVTVSS

SEQ ID NO: 20 - protein, 121 aa, Artificial Sequence
  DOMAIN: Variable region
EVQLLESGGGLVQPGGSLRLSCAASGFTVSNYWMNWVRQAPGKGLEWMGRIDPTDSETHYNQKFKDRVTISVDKSKNQFSLKLSSVTAADTAVYYCARSGFGSTYWFFDVWGQGTTVTVSS

SEQ ID NO: 21 - protein, 451 aa, Artificial Sequence
  CHAIN: Heavy chain
EVQLLESGGGLVQPGGSLRLSCAASGFTVSNYWMNWVRQAPGKGLEWMGRIDPRDSETHYNQKFKDRVTISVDKSKNQFSLKLSSVTAADTAVYYCARSGFGSTYWFFDVWGQGTTVTVSSASTKGPSVFPLAPSSKSTSGGTAALGCLVKDYFPEPVTVSWNSGALTSGVHTFPAVLQSSGLYSLSSVVTVPSSSLGTQTYICNVNHKPSNTKVDKKVEPKSCDKTHTCPPCPAPELLGGPSVFLFPPKPKDTLMISRTPEVTCVVVDVSHEDPEVKFNWYVDGVEVHNAKTKPREEQYNSTYRVVSVLTVLHQDWLNGKEYKCKVSNKALPAPIEKTISKAKGQPREPQVYTLPPSRDELTKNQVSLTCLVKGFYPSDIAVEWESNGQPENNYKTTPPVLDSDGSFFLYSKLTVDKSRWQQGNVFSCSVMHEALHNHYTQKSLSLSPGK

SEQ ID NO: 22 - protein, 451 aa, Artificial Sequence
  CHAIN: Heavy chain
EVQLLESGGGLVQPGGSLRLSCAASGFTVSNYWMNWVRQAPGKGLEWMGRIDPYDSETHYNQKFKDRVTISVDKSKNQFSLKLSSVTAADTAVYYCARSGFGSTYWFFDVWGQGTTVTVSSASTKGPSVFPLAPSSKSTSGGTAALGCLVKDYFPEPVTVSWNSGALTSGVHTFPAVLQSSGLYSLSSVVTVPSSSLGTQTYICNVNHKPSNTKVDKKVEPKSCDKTHTCPPCPAPELLGGPSVFLFPPKPKDTLMISRTPEVTCVVVDVSHEDPEVKFNWYVDGVEVHNAKTKPREEQYNSTYRVVSVLTVLHQDWLNGKEYKCKVSNKALPAPIEKTISKAKGQPREPQVYTLPPSRDELTKNQVSLTCLVKGFYPSDIAVEWESNGQPENNYKTTPPVLDSDGSFFLYSKLTVDKSRWQQGNVFSCSVMHEALHNHYTQKSLSLSPGK

SEQ ID NO: 23 - protein, 451 aa, Artificial Sequence
  CHAIN: Heavy chain
EVQLLESGGGLVQPGGSLRLSCAASGFTVSNYWMNWVRQAPGKGLEWMGRIDPQDSETHYNQKFKDRVTISVDKSKNQFSLKLSSVTAADTAVYYCARSGFGSTYWFFDVWGQGTTVTVSSASTKGPSVFPLAPSSKSTSGGTAALGCLVKDYFPEPVTVSWNSGALTSGVHTFPAVLQSSGLYSLSSVVTVPSSSLGTQTYICNVNHKPSNTKVDKKVEPKSCDKTHTCPPCPAPELLGGPSVFLFPPKPKDTLMISRTPEVTCVVVDVSHEDPEVKFNWYVDGVEVHNAKTKPREEQYNSTYRVVSVLTVLHQDWLNGKEYKCKVSNKALPAPIEKTISKAKGQPREPQVYTLPPSRDELTKNQVSLTCLVKGFYPSDIAVEWESNGQPENNYKTTPPVLDSDGSFFLYSKLTVDKSRWQQGNVFSCSVMHEALHNHYTQKSLSLSPGK

SEQ ID NO: 24 - protein, 451 aa, Artificial Sequence
  CHAIN: Heavy chain
EVQLLESGGGLVQPGGSLRLSCAASGFTVSNYWMNWVRQAPGKGLEWMGRIDPLDSETHYNQKFKDRVTISVDKSKNQFSLKLSSVTAADTAVYYCARSGFGSTYWFFDVWGQGTTVTVSSASTKGPSVFPLAPSSKSTSGGTAALGCLVKDYFPEPVTVSWNSGALTSGVHTFPAVLQSSGLYSLSSVVTVPSSSLGTQTYICNVNHKPSNTKVDKKVEPKSCDKTHTCPPCPAPELLGGPSVFLFPPKPKDTLMISRTPEVTCVVVDVSHEDPEVKFNWYVDGVEVHNAKTKPREEQYNSTYRVVSVLTVLHQDWLNGKEYKCKVSNKALPAPIEKTISKAKGQPREPQVYTLPPSRDELTKNQVSLTCLVKGFYPSDIAVEWESNGQPENNYKTTPPVLDSDGSFFLYSKLTVDKSRWQQGNVFSCSVMHEALHNHYTQKSLSLSPGK

SEQ ID NO: 25 - protein, 451 aa, Artificial Sequence
  CHAIN: Heavy chain
EVQLLESGGGLVQPGGSLRLSCAASGFTVSNYWMNWVRQAPGKGLEWMGRIDPTDSETHYNQKFKDRVTISVDKSKNQFSLKLSSVTAADTAVYYCARSGFGSTYWFFDVWGQGTTVTVSSASTKGPSVFPLAPSSKSTSGGTAALGCLVKDYFPEPVTVSWNSGALTSGVHTFPAVLQSSGLYSLSSVVTVPSSSLGTQTYICNVNHKPSNTKVDKKVEPKSCDKTHTCPPCPAPELLGGPSVFLFPPKPKDTLMISRTPEVTCVVVDVSHEDPEVKFNWYVDGVEVHNAKTKPREEQYNSTYRVVSVLTVLHQDWLNGKEYKCKVSNKALPAPIEKTISKAKGQPREPQVYTLPPSRDELTKNQVSLTCLVKGFYPSDIAVEWESNGQPENNYKTTPPVLDSDGSFFLYSKLTVDKSRWQQGNVFSCSVMHEALHNHYTQKSLSLSPGK

SEQ ID NO: 26 - protein, 17 aa, Artificial Sequence
  DOMAIN: CDR
RIDPRDSETHYNQKFKD

SEQ ID NO: 27 - protein, 17 aa, Artificial Sequence
  DOMAIN: CDR
RIDPYDSETHYNQKFKD

SEQ ID NO: 28 - protein, 17 aa, Artificial Sequence
  DOMAIN: CDR
RIDPQDSETHYNQKFKD

SEQ ID NO: 29 - protein, 17 aa, Artificial Sequence
  DOMAIN: CDR
RIDPLDSETHYNQKFKD

SEQ ID NO: 30 - protein, 17 aa, Artificial Sequence
  DOMAIN: CDR
RIDPTDSETHYNQKFKD

SEQ ID NO: 31 - protein, 121 aa, Artificial Sequence
  DOMAIN: Variable region
EVQLLESGGGLVQPGGSLRLSCAASGFTVSNYWMNWVRQAPGKGLEWMGRIDPIDSETHYNQKFKDRVTISVDKSKNQFSLKLSSVTAADTAVYYCARSGFGSTYWFFDVWGQGTTVTVSS

SEQ ID NO: 32 - protein, 121 aa, Artificial Sequence
  DOMAIN: Variable region
EVQLLESGGGLVQPGGSLRLSCAASGFTVSNYWMNWVRQAPGKGLEWMGRIDPFDSETHYNQKFKDRVTISVDKSKNQFSLKLSSVTAADTAVYYCARSGFGSTYWFFDVWGQGTTVTVSS

SEQ ID NO: 33 - protein, 121 aa, Artificial Sequence
  DOMAIN: Variable region
EVQLLESGGGLVQPGGSLRLSCAASGFTVSNYWMNWVRQAPGKGLEWMGRIDPEDSETHYNQKFKDRVTISVDKSKNQFSLKLSSVTAADTAVYYCARSGFGSTYWFFDVWGQGTTVTVSS

SEQ ID NO: 34 - protein, 121 aa, Artificial Sequence
  DOMAIN: Variable region
EVQLLESGGGLVQPGGSLRLSCAASGFTVSNYWMNWVRQAPGKGLEWMGRIDPADSETHYNQKFKDRVTISVDKSKNQFSLKLSSVTAADTAVYYCARSGFGSTYWFFDVWGQGTTVTVSS

SEQ ID NO: 35 - protein, 451 aa, Artificial Sequence
  CHAIN: Heavy chain
EVQLLESGGGLVQPGGSLRLSCAASGFTVSNYWMNWVRQAPGKGLEWMGRIDPIDSETHYNQKFKDRVTISVDKSKNQFSLKLSSVTAADTAVYYCARSGFGSTYWFFDVWGQGTTVTVSSASTKGPSVFPLAPSSKSTSGGTAALGCLVKDYFPEPVTVSWNSGALTSGVHTFPAVLQSSGLYSLSSVVTVPSSSLGTQTYICNVNHKPSNTKVDKKVEPKSCDKTHTCPPCPAPELLGGPSVFLFPPKPKDTLMISRTPEVTCVVVDVSHEDPEVKFNWYVDGVEVHNAKTKPREEQYNSTYRVVSVLTVLHQDWLNGKEYKCKVSNKALPAPIEKTISKAKGQPREPQVYTLPPSRDELTKNQVSLTCLVKGFYPSDIAVEWESNGQPENNYKTTPPVLDSDGSFFLYSKLTVDKSRWQQGNVFSCSVMHEALHNHYTQKSLSLSPGK

SEQ ID NO: 36 - protein, 451 aa, Artificial Sequence
  CHAIN: Heavy chain
EVQLLESGGGLVQPGGSLRLSCAASGFTVSNYWMNWVRQAPGKGLEWMGRIDPFDSETHYNQKFKDRVTISVDKSKNQFSLKLSSVTAADTAVYYCARSGFGSTYWFFDVWGQGTTVTVSSASTKGPSVFPLAPSSKSTSGGTAALGCLVKDYFPEPVTVSWNSGALTSGVHTFPAVLQSSGLYSLSSVVTVPSSSLGTQTYICNVNHKPSNTKVDKKVEPKSCDKTHTCPPCPAPELLGGPSVFLFPPKPKDTLMISRTPEVTCVVVDVSHEDPEVKFNWYVDGVEVHNAKTKPREEQYNSTYRVVSVLTVLHQDWLNGKEYKCKVSNKALPAPIEKTISKAKGQPREPQVYTLPPSRDELTKNQVSLTCLVKGFYPSDIAVEWESNGQPENNYKTTPPVLDSDGSFFLYSKLTVDKSRWQQGNVFSCSVMHEALHNHYTQKSLSLSPGK

SEQ ID NO: 37 - protein, 451 aa, Artificial Sequence
  CHAIN: Heavy chain
EVQLLESGGGLVQPGGSLRLSCAASGFTVSNYWMNWVRQAPGKGLEWMGRIDPEDSETHYNQKFKDRVTISVDKSKNQFSLKLSSVTAADTAVYYCARSGFGSTYWFFDVWGQGTTVTVSSASTKGPSVFPLAPSSKSTSGGTAALGCLVKDYFPEPVTVSWNSGALTSGVHTFPAVLQSSGLYSLSSVVTVPSSSLGTQTYICNVNHKPSNTKVDKKVEPKSCDKTHTCPPCPAPELLGGPSVFLFPPKPKDTLMISRTPEVTCVVVDVSHEDPEVKFNWYVDGVEVHNAKTKPREEQYNSTYRVVSVLTVLHQDWLNGKEYKCKVSNKALPAPIEKTISKAKGQPREPQVYTLPPSRDELTKNQVSLTCLVKGFYPSDIAVEWESNGQPENNYKTTPPVLDSDGSFFLYSKLTVDKSRWQQGNVFSCSVMHEALHNHYTQKSLSLSPGK

SEQ ID NO: 38 - protein, 451 aa, Artificial Sequence
  CHAIN: Heavy chain
EVQLLESGGGLVQPGGSLRLSCAASGFTVSNYWMNWVRQAPGKGLEWMGRIDPADSETHYNQKFKDRVTISVDKSKNQFSLKLSSVTAADTAVYYCARSGFGSTYWFFDVWGQGTTVTVSSASTKGPSVFPLAPSSKSTSGGTAALGCLVKDYFPEPVTVSWNSGALTSGVHTFPAVLQSSGLYSLSSVVTVPSSSLGTQTYICNVNHKPSNTKVDKKVEPKSCDKTHTCPPCPAPELLGGPSVFLFPPKPKDTLMISRTPEVTCVVVDVSHEDPEVKFNWYVDGVEVHNAKTKPREEQYNSTYRVVSVLTVLHQDWLNGKEYKCKVSNKALPAPIEKTISKAKGQPREPQVYTLPPSRDELTKNQVSLTCLVKGFYPSDIAVEWESNGQPENNYKTTPPVLDSDGSFFLYSKLTVDKSRWQQGNVFSCSVMHEALHNHYTQKSLSLSPGK

SEQ ID NO: 39 - protein, 17 aa, Artificial Sequence
  DOMAIN: CDR
RIDPIDSETHYNQKFKD

SEQ ID NO: 40 - protein, 17 aa, Artificial Sequence
  DOMAIN: CDR
RIDPFDSETHYNQKFKD

SEQ ID NO: 41 - protein, 17 aa, Artificial Sequence
  DOMAIN: CDR
RIDPEDSETHYNQKFKD

SEQ ID NO: 42 - protein, 17 aa, Artificial Sequence
  DOMAIN: CDR
RIDPADSETHYNQKFKD

SEQ ID NO: 43 - protein, 17 aa, Artificial Sequence
  VARIANT (5)..(5): X is selected from the group consisting of R, Y, Q, L, T, I, F, E and A
  DOMAIN: CDR
RIDPXDSETHYNQKFKD